European Patent Application EP 4 242 663 A2, published September 13, 2023. Title: METHODS FOR CHARACTERIZING COMPOSITIONS COMPRISING PEANUT ANTIGENS. Applicant: Sanofi. Application EP. The sequence listing filed with the application follows.

SEQUENCE LISTING (253 sequences)

SEQ ID NO: 1 - protein, 14 aa, Arachis hypogaea
ACESRCTKLEYDPR

SEQ ID NO: 2 - protein, 20 aa, Arachis hypogaea
ACESRCTKLEYDPRCVYDPR

SEQ ID NO: 3 - protein, 9 aa, Arachis hypogaea
AMVIVVVNK

SEQ ID NO: 4 - protein, 20 aa, Arachis hypogaea
AMVIVVVNKGTGNLELVAVR

SEQ ID NO: 5 - protein, 21 aa, Arachis hypogaea
AMVIVVVNKGTGNLELVAVRK

SEQ ID NO: 6 - protein, 13 aa, Arachis hypogaea
CLQSCQQEPDDLK

SEQ ID NO: 7 - protein, 15 aa, Arachis hypogaea
CLQSCQQEPDDLKQK

SEQ ID NO: 8 - protein, 20 aa, Arachis hypogaea
CLQSCQQEPDDLKQKACESR

SEQ ID NO: 9 - protein, 23 aa, Arachis hypogaea
CLQSCQQEPDDLKQKACESRCTK

SEQ ID NO: 10 - protein, 9 aa, Arachis hypogaea
CTKLEYDPR

SEQ ID NO: 11 - protein, 15 aa, Arachis hypogaea
CTKLEYDPRCVYDPR

SEQ ID NO: 12 - protein, 24 aa, Arachis hypogaea
CTKLEYDPRCVYDPRGHTGTTNQR

SEQ ID NO: 13 - protein, 6 aa, Arachis hypogaea
CVYDPR

SEQ ID NO: 14 - protein, 15 aa, Arachis hypogaea
CVYDPRGHTGTTNQR

SEQ ID NO: 15 - protein, 21 aa, Arachis hypogaea
CVYDPRGHTGTTNQRSPPGER

SEQ ID NO: 16 - protein, 23 aa, Arachis hypogaea
CVYDPRGHTGTTNQRSPPGERTR

SEQ ID NO: 17 - protein, 13 aa, Arachis hypogaea
DLAFPGSGEQVEK

SEQ ID NO: 18 - protein, 16 aa, Arachis hypogaea
DLAFPGSGEQVEKLIK

SEQ ID NO: 19 - protein, 12 aa, Arachis hypogaea
DNVIDQIEKQAK

SEQ ID NO: 20 - protein, 11 aa, Arachis hypogaea
DQSSYLQGFSR

SEQ ID NO: 21 - protein, 27 aa, Arachis hypogaea
DQSSYLQGFSRNTLEAAFNAEFNEIRR

SEQ ID NO: 22 - protein, 19 aa, Arachis hypogaea
EDQEEENQGGKGPLLSILK

SEQ ID NO: 23 - protein, 12 aa, Arachis hypogaea
EDWRRPSHQQPR

SEQ ID NO: 24 - protein, 12 aa, Arachis hypogaea
EEDWRQPREDWR

SEQ ID NO: 25 - protein, 20 aa, Arachis hypogaea
EEDWRQPREDWRRPSHQQPR

SEQ ID NO: 26 - protein, 23 aa, Arachis hypogaea
EEEEDEDEEEEGSNREVRRYTAR

SEQ ID NO: 27 - protein, 12 aa, Arachis hypogaea
EEGGRWGPAGPR

SEQ ID NO: 28 - protein, 14 aa, Arachis hypogaea
EEGGRWGPAGPRER

SEQ ID NO: 29 - protein, 16 aa, Arachis hypogaea
EEGGRWGPAGPRERER

SEQ ID NO: 30 - protein, 14 aa, Arachis hypogaea
EETSRNNPFYFPSR

SEQ ID NO: 31 - protein, 15 aa, Arachis hypogaea
EETSRNNPFYFPSRR

SEQ ID NO: 32 - protein, 19 aa, Arachis hypogaea
EETSRNNPFYFPSRRFSTR

SEQ ID NO: 33 - protein, 12 aa, Arachis hypogaea
EGALMLPHFNSK

SEQ ID NO: 34 - protein, 21 aa, Arachis hypogaea
EGALMLPHFNSKAMVIVVVNK

SEQ ID NO: 35 - protein, 42 aa, Arachis hypogaea
EGDVFIMPAAHPVAINASSELHLLGFGINAENNHRIFLAGDK

SEQ ID NO: 36 - protein, 51 aa, Arachis hypogaea
EGDVFIMPAAHPVAINASSELHLLGFGINAENNHRIFLAGDKDNVIDQIEK

SEQ ID NO: 37 - protein, 12 aa, Arachis hypogaea
EGEPDLSNNFGK

SEQ ID NO: 38 - protein, 21 aa, Arachis hypogaea
EGEPDLSNNFGKLFEVKPDKK

SEQ ID NO: 39 - protein, 38 aa, Arachis hypogaea
EGEPDLSNNFGKLFEVKPDKKNPQLQDLDMMLTCVEIK

SEQ ID NO: 40 - protein, 14 aa, Arachis hypogaea
EGEQEWGTPGSHVR

SEQ ID NO: 41 - protein, 29 aa, Arachis hypogaea
EGEQEWGTPGSHVREETSRNNPFYFPSRR

SEQ ID NO: 42 - protein, 8 aa, Arachis hypogaea
EHVEELTK

SEQ ID NO: 43 - protein, 11 aa, Arachis hypogaea
EHVEELTKHAK

SEQ ID NO: 44 - protein, 8 aa, Arachis hypogaea
EQQQRGRR

SEQ ID NO: 45 - protein, 23 aa, Arachis hypogaea
EQQQRGRREEEEDEDEEEEGSNR

SEQ ID NO: 46 - protein, 7 aa, Arachis hypogaea
EREEDWR

SEQ ID NO: 47 - protein, 10 aa, Arachis hypogaea
EREEDWRQPR

SEQ ID NO: 48 - protein, 9 aa, Arachis hypogaea
EREREEDWR

SEQ ID NO: 49 - protein, 12 aa, Arachis hypogaea
EREREEDWRQPR

SEQ ID NO: 50 - protein, 21 aa, Arachis hypogaea
ESHFVSARPQSQSQSPSSPEK

SEQ ID NO: 51 - protein, 37 aa, Arachis hypogaea
ESHFVSARPQSQSQSPSSPEKESPEKEDQEEENQGGK

SEQ ID NO: 52 - protein, 16 aa, Arachis hypogaea
ESPEKEDQEEENQGGK

SEQ ID NO: 53 - protein, 8 aa, Arachis hypogaea
EVRRYTAR

SEQ ID NO: 54 - protein, 6 aa, Arachis hypogaea
FDQRSR

SEQ ID NO: 55 - protein, 15 aa, Arachis hypogaea
FDQRSRQFQNLQNHR

SEQ ID NO: 56 - protein, 11 aa, Arachis hypogaea
FSTRYGNQNGR

SEQ ID NO: 57 - protein, 13 aa, Arachis hypogaea
FSTRYGNQNGRIR

SEQ ID NO: 58 - protein, 13 aa, Arachis hypogaea
FSTRYGNQNGRIR

SEQ ID NO: 59 - protein, 17 aa, Arachis hypogaea
GHTGTTNQRSPPGERTR

SEQ ID NO: 60 - protein, 19 aa, Arachis hypogaea
GHTGTTNQRSPPGERTRGR

SEQ ID NO: 61 - protein, 8 aa, Arachis hypogaea
GQRRWSTR

SEQ ID NO: 62 - protein, 11 aa, Arachis hypogaea
GRQPGDYDDDR

SEQ ID NO: 63 - protein, 12 aa, Arachis hypogaea
GRQPGDYDDDRR

SEQ ID NO: 64 - protein, 15 aa, Arachis hypogaea
GRQPGDYDDDRRQPR

SEQ ID NO: 65 - protein, 15 aa, Arachis hypogaea
GRQPGDYDDDRRQPR

SEQ ID NO: 66 - protein, 18 aa, Arachis hypogaea
GRREEEEDEDEEEEGSNR

SEQ ID NO: 67 - protein, 21 aa, Arachis hypogaea
GRREEEEDEDEEEEGSNREVR

SEQ ID NO: 68 - protein, 15 aa, Arachis hypogaea
GSEEEGDITNPINLR

SEQ ID NO: 69 - protein, 27 aa, Arachis hypogaea
GSEEEGDITNPINLREGEPDLSNNFGK

SEQ ID NO: 70 - protein, 11 aa, Arachis hypogaea
GTGNLELVAVR

SEQ ID NO: 71 - protein, 12 aa, Arachis hypogaea
GTGNLELVAVRK

SEQ ID NO: 72 - protein, 25 aa, Arachis hypogaea
HADADNILVIQQGQATVTVANGNNR

SEQ ID NO: 73 - protein, 26 aa, Arachis hypogaea
HADADNILVIQQGQATVTVANGNNRK

SEQ ID NO: 74 - protein, 37 aa, Arachis hypogaea
HADADNILVIQQGQATVTVANGNNRKSFNLDEGHALR

SEQ ID NO: 75 - protein, 8 aa, Arachis hypogaea
HAKSVSKK

SEQ ID NO: 76 - protein, 23 aa, Arachis hypogaea
HAKSVSKKGSEEEGDITNPINLR

SEQ ID NO: 77 - protein, 7 aa, Arachis hypogaea
HDNQNLR

SEQ ID NO: 78 - protein, 30 aa, Arachis hypogaea
HDNQNLRVAKISMPVNTPGQFEDFFPASSR

SEQ ID NO: 79 - protein, 16 aa, Arachis hypogaea
IFLAGDKDNVIDQIEK

SEQ ID NO: 80 - protein, 19 aa, Arachis hypogaea
IFLAGDKDNVIDQIEKQAK

SEQ ID NO: 81 - protein, 32 aa, Arachis hypogaea
IFLAGDKDNVIDQIEKQAKDLAFPGSGEQVEK

SEQ ID NO: 82 - protein, 12 aa, Arachis hypogaea
IPSGFISYILNR

SEQ ID NO: 83 - protein, 19 aa, Arachis hypogaea
IPSGFISYILNRHDNQNLR

SEQ ID NO: 84 - protein, 22 aa, Arachis hypogaea
IPSGFISYILNRHDNQNLRVAK

SEQ ID NO: 85 - protein, 42 aa, Arachis hypogaea
IPSGFISYILNRHDNQNLRVAKISMPVNTPGQFEDFFPASSR

SEQ ID NO: 86 - protein, 25 aa, Arachis hypogaea
IRPEGREGEQEWGTPGSHVREETSR

SEQ ID NO: 87 - protein, 34 aa, Arachis hypogaea
IRPEGREGEQEWGTPGSHVREETSRNNPFYFPSR

SEQ ID NO: 88 - protein, 10 aa, Arachis hypogaea
IRVLQRFDQR

SEQ ID NO: 89 - protein, 20 aa, Arachis hypogaea
ISMPVNTPGQFEDFFPASSR

SEQ ID NO: 90 - protein, 31 aa, Arachis hypogaea
ISMPVNTPGQFEDFFPASSRDQSSYLQGFSR

SEQ ID NO: 91 - protein, 46 aa, Arachis hypogaea
ISMPVNTPGQFEDFFPASSRDQSSYLQGFSRNTLEAAFNAEFNEIR

SEQ ID NO: 92 - protein, 47 aa, Arachis hypogaea
ISMPVNTPGQFEDFFPASSRDQSSYLQGFSRNTLEAAFNAEFNEIRR

SEQ ID NO: 93 - protein, 15 aa, Arachis hypogaea
IVQIEAKPNTLVLPK

SEQ ID NO: 94 - protein, 6 aa, Arachis hypogaea
KEQQQR

SEQ ID NO: 95 - protein, 9 aa, Arachis hypogaea
KEQQQRGRR

SEQ ID NO: 96 - protein, 16 aa, Arachis hypogaea
KGSEEEGDITNPINLR

SEQ ID NO: 97 - protein, 28 aa, Arachis hypogaea
KGSEEEGDITNPINLREGEPDLSNNFGK

SEQ ID NO: 98 - protein, 36 aa, Arachis hypogaea
KGSEEEGDITNPINLREGEPDLSNNFGKLFEVKPDK

SEQ ID NO: 99 - protein, 26 aa, Arachis hypogaea
KIRPEGREGEQEWGTPGSHVREETSR

SEQ ID NO: 100 - protein, 18 aa, Arachis hypogaea
KNPQLQDLDMMLTCVEIK

SEQ ID NO: 101 - protein, 30 aa, Arachis hypogaea
KNPQLQDLDMMLTCVEIKEGALMLPHFNSK

SEQ ID NO: 102 - protein, 39 aa, Arachis hypogaea
KNPQLQDLDMMLTCVEIKEGALMLPHFNSKAMVIVVVNK

SEQ ID NO: 103 - protein, 12 aa, Arachis hypogaea
KSFNLDEGHALR

SEQ ID NO: 104 - protein, 24 aa, Arachis hypogaea
KSFNLDEGHALRIPSGFISYILNR

SEQ ID NO: 105 - protein, 31 aa, Arachis hypogaea
KSFNLDEGHALRIPSGFISYILNRHDNQNLR

SEQ ID NO: 106 - protein, 9 aa, Arachis hypogaea
KTENPCAQR

SEQ ID NO: 107 - protein, 22 aa, Arachis hypogaea
KTENPCAQRCLQSCQQEPDDLK

SEQ ID NO: 108 - protein, 24 aa, Arachis hypogaea
KTENPCAQRCLQSCQQEPDDLKQK

SEQ ID NO: 109 - protein, 6 aa, Arachis hypogaea
LEYDPR

SEQ ID NO: 110 - protein, 12 aa, Arachis hypogaea
LEYDPRCVYDPR

SEQ ID NO: 111 - protein, 21 aa, Arachis hypogaea
LEYDPRCVYDPRGHTGTTNQR

SEQ ID NO: 112 - protein, 27 aa, Arachis hypogaea
LEYDPRCVYDPRGHTGTTNQRSPPGER

SEQ ID NO: 113 - protein, 8 aa, Arachis hypogaea
LFEVKPDK

SEQ ID NO: 114 - protein, 9 aa, Arachis hypogaea
LFEVKPDKK

SEQ ID NO: 115 - protein, 26 aa, Arachis hypogaea
LFEVKPDKKNPQLQDLDMMLTCVEIK

SEQ ID NO: 116 - protein, 38 aa, Arachis hypogaea
LFEVKPDKKNPQLQDLDMMLTCVEIKEGALMLPHFNSK

SEQ ID NO: 117 - protein, 27 aa, Arachis hypogaea
LIKNQKESHFVSARPQSQSQSPSSPEK

SEQ ID NO: 118 - protein, 9 aa, Arachis hypogaea
NNPFYFPSR

SEQ ID NO: 119 - protein, 10 aa, Arachis hypogaea
NNPFYFPSRR

SEQ ID NO: 120 - protein, 14 aa, Arachis hypogaea
NNPFYFPSRRFSTR

SEQ ID NO: 121 - protein, 21 aa, Arachis hypogaea
NNPFYFPSRRFSTRYGNQNGR

SEQ ID NO: 122 - protein, 17 aa, Arachis hypogaea
NPQLQDLDMMLTCVEIK

SEQ ID NO: 123 - protein, 29 aa, Arachis hypogaea
NPQLQDLDMMLTCVEIKEGALMLPHFNSK

SEQ ID NO: 124 - protein, 38 aa, Arachis hypogaea
NPQLQDLDMMLTCVEIKEGALMLPHFNSKAMVIVVVNK

SEQ ID NO: 125 - protein, 24 aa, Arachis hypogaea
NQKESHFVSARPQSQSQSPSSPEK

SEQ ID NO: 126 - protein, 40 aa, Arachis hypogaea
NQKESHFVSARPQSQSQSPSSPEKESPEKEDQEEENQGGK

SEQ ID NO: 127 - protein, 15 aa, Arachis hypogaea
NTLEAAFNAEFNEIR

SEQ ID NO: 128 - protein, 16 aa, Arachis hypogaea
NTLEAAFNAEFNEIRR

SEQ ID NO: 129 - protein, 30 aa, Arachis hypogaea
NTLEAAFNAEFNEIRRVLLEENAGGEQEER

SEQ ID NO: 130 - protein, 33 aa, Arachis hypogaea
NTLEAAFNAEFNEIRRVLLEENAGGEQEERGQR

SEQ ID NO: 131 - protein, 16 aa, Arachis hypogaea
QAKDLAFPGSGEQVEK

SEQ ID NO: 132 - protein, 9 aa, Arachis hypogaea
QFQNLQNHR

SEQ ID NO: 133 - protein, 50 aa, Arachis hypogaea
QFQNLQNHRIVQIEAKPNTLVLPKHADADNILVIQQGQATVTVANGNNRK

SEQ ID NO: 134 - protein, 7 aa, Arachis hypogaea
QKACESR

SEQ ID NO: 135 - protein, 16 aa, Arachis hypogaea
QKACESRCTKLEYDPR

SEQ ID NO: 136 - protein, 10 aa, Arachis hypogaea
QPGDYDDDRR

SEQ ID NO: 137 - protein, 13 aa, Arachis hypogaea
QPGDYDDDRRQPR

SEQ ID NO: 138 - protein, 14 aa, Arachis hypogaea
QPGDYDDDRRQPRR

SEQ ID NO: 139 - protein, 15 aa, Arachis hypogaea
QPREDWRRPSHQQPR

SEQ ID NO: 140 - protein, 16 aa, Arachis hypogaea
QPREDWRRPSHQQPRK

SEQ ID NO: 141 - protein, 9 aa, Arachis hypogaea
QPRREEGGR

SEQ ID NO: 142 - protein, 16 aa, Arachis hypogaea
QPRREEGGRWGPAGPR

SEQ ID NO: 143 - protein, 16 aa, Arachis hypogaea
REEEEDEDEEEEGSNR

SEQ ID NO: 144 - protein, 19 aa, Arachis hypogaea
REEEEDEDEEEEGSNREVR

SEQ ID NO: 145 - protein, 20 aa, Arachis hypogaea
REEEEDEDEEEEGSNREVRR

SEQ ID NO: 146 - protein, 6 aa, Arachis hypogaea
REEGGR

SEQ ID NO: 147 - protein, 13 aa, Arachis hypogaea
REEGGRWGPAGPR

SEQ ID NO: 148 - protein, 15 aa, Arachis hypogaea
REEGGRWGPAGPRER

SEQ ID NO: 149 - protein, 12 aa, Arachis hypogaea
RFSTRYGNQNGR

SEQ ID NO: 150 - protein, 14 aa, Arachis hypogaea
RFSTRYGNQNGRIR

SEQ ID NO: 151 - protein, 8 aa, Arachis hypogaea
RPSHQQPR

SEQ ID NO: 152 - protein, 15 aa, Arachis hypogaea
RVLLEENAGGEQEER

SEQ ID NO: 153 - protein, 18 aa, Arachis hypogaea
RVLLEENAGGEQEERGQR

SEQ ID NO: 154 - protein, 16 aa, Arachis hypogaea
RWSTRSSENNEGVIVK

SEQ ID NO: 155 - protein, 11 aa, Arachis hypogaea
SFNLDEGHALR

SEQ ID NO: 156 - protein, 23 aa, Arachis hypogaea
SFNLDEGHALRIPSGFISYILNR

SEQ ID NO: 157 - protein, 30 aa, Arachis hypogaea
SFNLDEGHALRIPSGFISYILNRHDNQNLR

SEQ ID NO: 158 - protein, 10 aa, Arachis hypogaea
SPPGERTRGR

SEQ ID NO: 159 - protein, 19 aa, Arachis hypogaea
SPPGERTRGRQPGDYDDDR

SEQ ID NO: 160 - protein, 11 aa, Arachis hypogaea
SRQFQNLQNHR

SEQ ID NO: 161 - protein, 51 aa, Arachis hypogaea
SRQFQNLQNHRIVQIEAKPNTLVLPKHADADNILVIQQGQATVTVANGNNR

SEQ ID NO: 162 - protein, 11 aa, Arachis hypogaea
SSENNEGVIVK

SEQ ID NO: 163 - protein, 14 aa, Arachis hypogaea
SSENNEGVIVKVSK

SEQ ID NO: 164 - protein, 22 aa, Arachis hypogaea
SSENNEGVIVKVSKEHVEELTK

SEQ ID NO: 165 - protein, 7 aa, Arachis hypogaea
SSPYQKK

SEQ ID NO: 166 - protein, 15 aa, Arachis hypogaea
SSPYQKKTENPCAQR

SEQ ID NO: 167 - protein, 28 aa, Arachis hypogaea
SSPYQKKTENPCAQRCLQSCQQEPDDLK

SEQ ID NO: 168 - protein, 20 aa, Arachis hypogaea
SVSKKGSEEEGDITNPINLR

SEQ ID NO: 169 - protein, 8 aa, Arachis hypogaea
TENPCAQR

SEQ ID NO: 170 - protein, 21 aa, Arachis hypogaea
TENPCAQRCLQSCQQEPDDLK

SEQ ID NO: 171 - protein, 23 aa, Arachis hypogaea
TENPCAQRCLQSCQQEPDDLKQK

SEQ ID NO: 172 - protein, 28 aa, Arachis hypogaea
TENPCAQRCLQSCQQEPDDLKQKACESR

SEQ ID NO: 173 - protein, 13 aa, Arachis hypogaea
TRGRQPGDYDDDR

SEQ ID NO: 174 - protein, 14 aa, Arachis hypogaea
TRGRQPGDYDDDRR

SEQ ID NO: 175 - protein, 23 aa, Arachis hypogaea
VAKISMPVNTPGQFEDFFPASSR

SEQ ID NO: 176 - protein, 49 aa, Arachis hypogaea
VAKISMPVNTPGQFEDFFPASSRDQSSYLQGFSRNTLEAAFNAEFNEIR

SEQ ID NO: 177 - protein, 14 aa, Arachis hypogaea
VLLEENAGGEQEER

SEQ ID NO: 178 - protein, 17 aa, Arachis hypogaea
VLLEENAGGEQEERGQR

SEQ ID NO: 179 - protein, 18 aa, Arachis hypogaea
VLLEENAGGEQEERGQRR

SEQ ID NO: 180 - protein, 22 aa, Arachis hypogaea
VLLEENAGGEQEERGQRRWSTR

SEQ ID NO: 181 - protein, 19 aa, Arachis hypogaea
VLQRFDQRSRQFQNLQNHR

SEQ ID NO: 182 - protein, 11 aa, Arachis hypogaea
VSKEHVEELTK

SEQ ID NO: 183 - protein, 22 aa, Arachis hypogaea
VSPLMLLLGILVLASVSATHAK

SEQ ID NO: 184 - protein, 7 aa, Arachis hypogaea
WGPAGPR

SEQ ID NO: 185 - protein, 9 aa, Arachis hypogaea
WGPAGPRER

SEQ ID NO: 186 - protein, 11 aa, Arachis hypogaea
WGPAGPRERER

SEQ ID NO: 187 - protein, 15 aa, Arachis hypogaea
WSTRSSENNEGVIVK

SEQ ID NO: 188 - protein, 26 aa, Arachis hypogaea
WSTRSSENNEGVIVKVSKEHVEELTK

SEQ ID NO: 189 - protein, 7 aa, Arachis hypogaea
YGNQNGR

SEQ ID NO: 190 - protein, 13 aa, Arachis hypogaea
YGNQNGRIRVLQR

SEQ ID NO: 191 - protein, 17 aa, Arachis hypogaea
YGNQNGRIRVLQRFDQR

SEQ ID NO: 192 - protein, 48 aa, Arachis hypogaea
YTARLKEGDVFIMPAAHPVAINASSELHLLGFGINAENNHRIFLAGDK

SEQ ID NO: 193 - protein, 18 aa, Arachis hypogaea
EQEWEEEEEDEEEEGSNR

SEQ ID NO: 194 - protein, 14 aa, Arachis hypogaea
GSEEEDITNPINLR

SEQ ID NO: 195 - protein, 14 aa, Arachis hypogaea
EGEQEWGTPGSEVR

SEQ ID NO: 196 - protein, 15 aa, Arachis hypogaea
IVQIEARPNTLVLPK

SEQ ID NO: 197 - protein, 10 aa, Arachis hypogaea
GAGSSQHQER

SEQ ID NO: 198 - protein, 7 aa, Arachis hypogaea
QQEQQFK

SEQ ID NO: 199 - protein, 17 aa, Arachis hypogaea
RPFYSNAPQEIFIQQGR

SEQ ID NO: 200 - protein, 12 aa, Arachis hypogaea
AHVQVVDSNGNR

SEQ ID NO: 201 - protein, 13 aa, Arachis hypogaea
FNLAGNHEQEFLR

SEQ ID NO: 202 - protein, 20 aa, Arachis hypogaea
NALFVPHYNTNAHSIIYALR

SEQ ID NO: 203 - protein, 13 aa, Arachis hypogaea
SPDIYNPQAGSLK

SEQ ID NO: 204 - protein, 13 aa, Arachis hypogaea
WLGLSAEYGNLYR

SEQ ID NO: 205 - protein, 23 aa, Arachis hypogaea
VYDEELQEGHVLVVPQNFAVAGK

SEQ ID NO: 206 - protein, 12 aa, Arachis hypogaea
SQSENFEYVAFK

SEQ ID NO: 207 - protein, 30 aa, Arachis hypogaea
AGQEQENEGGNIFSGFTPEFLAQAFQVDDR

SEQ ID NO: 208 - protein, 15 aa, Arachis hypogaea
GENESDEQGAIVTVR

SEQ ID NO: 209 - protein, 24 aa, Arachis hypogaea
QQYERPDEEEEYDEDEYEYDEEER

SEQ ID NO: 210 - protein, 12 aa, Arachis hypogaea
SQSDNFEYVAFK

SEQ ID NO: 211 - protein, 11 aa, Arachis hypogaea
TANDLNLLILR

SEQ ID NO: 212 - protein, 11 aa, Arachis hypogaea
TANELNLLILR

SEQ ID NO: 213 - protein, 33 aa, Arachis hypogaea
TDSRPSIANLAGENSFIDNLPEEVVANSYGLPR

SEQ ID NO: 214 - protein, 12 aa, Arachis hypogaea
AHVQVVDSNGDR

SEQ ID NO: 215 - protein, 12 aa, Arachis hypogaea
AQSENYEYLAFK

SEQ ID NO: 216 - protein, 45 aa, Arachis hypogaea
FNEGDLIAVPTGVAFWLYNDHDTDVVAVSLTDTNNNDNQLDQFPR

SEQ ID NO: 217 - protein, 20 aa, Arachis hypogaea
GADEEEEYDEDEYEYDEEDR

SEQ ID NO: 218 - protein, 15 aa, Arachis hypogaea
SSNPDIYNPQAGSLR

SEQ ID NO: 219 - protein, 24 aa, Arachis hypogaea
SVNELDLPILGWLGLSAQHGTIYR

SEQ ID NO: 220 - protein, 23 aa, Arachis hypogaea
VFDEELQEGHVLVVPQNFAVAGK

SEQ ID NO: 221 - protein, 23 aa, Arachis hypogaea
VYDEELQEGHVLVVPQNFAVAAK

SEQ ID NO: 222 - protein, 30 aa, Arachis hypogaea
AGQEEENEGGNIFSGFTPEFLAQAFQVDDR

SEQ ID NO: 223 - protein, 30 aa, Arachis hypogaea
AGQEEENEGGNIFSGFTPEFLEQAFQVDDR

SEQ ID NO: 224 - protein, 11 aa, Arachis hypogaea
FFVPPFQQSPR

SEQ ID NO: 225 - protein, 30 aa, Arachis hypogaea
TDSRPSIANLAGENSIIDNLPEEVVANSYR

SEQ ID NO: 226 - protein, 30 aa, Arachis hypogaea
AGQEEEDEGGNIFSGFTPEFLEQAFQVDDR

SEQ ID NO: 227 - protein, 30 aa, Arachis hypogaea
AGQEQENEGGNIFSGFTSEFLAQAFQVDDR

SEQ ID NO: 228 - protein, 15 aa, Arachis hypogaea
GENESEEEGAIVTVK

SEQ ID NO: 229 - protein, 15 aa, Arachis hypogaea
GENESEEQGAIVTVK

SEQ ID NO: 230 - protein, 18 aa, Arachis hypogaea
SPDEEEEYDEDEYAEEER

SEQ ID NO: 231 - protein, 12 aa, Arachis hypogaea
SQSEHFLYVAFK

SEQ ID NO: 232 - protein, 33 aa, Arachis hypogaea
TDSRPSIANLAGENSIIDNLPEEVVANSYGLPR

SEQ ID NO: 233 - protein, 33 aa, Arachis hypogaea
TDSRPSIANLAGENSVIDNLPEEVVANSYGLPR

SEQ ID NO: 234 - protein, 30 aa, Arachis hypogaea
TDSRPSIANQAGENSIIDNLPEEVVANSYR

SEQ ID NO: 235 - protein, 23 aa, Arachis hypogaea
VFDEELQEGQSLVVPQNFAVAAK

SEQ ID NO: 236 - protein, 14 aa, Arachis hypogaea
IMGEQEQYDSYDIR

SEQ ID NO: 237 - protein, 7 aa, Arachis hypogaea
QMVQQFK

SEQ ID NO: 238 - protein, 13 aa, synthetic construct
  REGION 1..13: note = source = /note="Description of Artificial Sequence: Synthetic peptide"
DLAFPGSGEQVEK

SEQ ID NO: 239 - protein, 11 aa, synthetic construct
  REGION 1..11: note = source = /note="Description of Artificial Sequence: Synthetic peptide"
GTGNLELVAVR

SEQ ID NO: 240 - protein, 10 aa, synthetic construct
  REGION 1..10: note = source = /note="Description of Artificial Sequence: Synthetic peptide"
GAGSSQHQER

SEQ ID NO: 241 - protein, 7 aa, synthetic construct
  REGION 1..7: note = source = /note="Description of Artificial Sequence: Synthetic peptide"
QQEQQFK

SEQ ID NO: 242 - protein, 17 aa, synthetic construct
  REGION 1..17: note = source = /note="Description of Artificial Sequence: Synthetic peptide"
RPFYSNAPQEIFIQQGR

SEQ ID NO: 243 - protein, 12 aa, synthetic construct
  REGION 1..12: note = source = /note="Description of Artificial Sequence: Synthetic peptide"
AHVQVVDSNGNR

SEQ ID NO: 244 - protein, 14 aa, synthetic construct
  REGION 1..14: note = source = /note="Description of Artificial Sequence: Synthetic peptide"
IMGEQEQYDSYDIR

SEQ ID NO: 245 - protein, 7 aa, synthetic construct
  REGION 1..7: note = source = /note="Description of Artificial Sequence: Synthetic peptide"
QMVQQFK

SEQ ID NO: 246 - protein, 13 aa, synthetic construct
  REGION 1..13: note = source = /note="Description of Artificial Sequence: Synthetic peptide"
DLAFPGSGEQVEK

SEQ ID NO: 247 - protein, 11 aa, synthetic construct
  REGION 1..11: note = source = /note="Description of Artificial Sequence: Synthetic peptide"
GTGNLELVAVR

SEQ ID NO: 248 - protein, 10 aa, synthetic construct
  REGION 1..10: note = source = /note="Description of Artificial Sequence: Synthetic peptide"
GAGSSQHQER

SEQ ID NO: 249 - protein, 7 aa, synthetic construct
  REGION 1..7: note = source = /note="Description of Artificial Sequence: Synthetic peptide"
QQEQQFK

SEQ ID NO: 250 - protein, 17 aa, synthetic construct
  REGION 1..17: note = source = /note="Description of Artificial Sequence: Synthetic peptide"
RPFYSNAPQEIFIQQGR

SEQ ID NO: 251 - protein, 12 aa, synthetic construct
  REGION 1..12: note = source = /note="Description of Artificial Sequence: Synthetic peptide"
AHVQVVDSNGNR

SEQ ID NO: 252 - protein, 14 aa, synthetic construct
  REGION 1..14: note = source = /note="Description of Artificial Sequence: Synthetic peptide"
IMGEQEQYDSYDIR

SEQ ID NO: 253 - protein, 7 aa, synthetic construct
  REGION 1..7: note = source = /note="Description of Artificial Sequence: Synthetic peptide"
QMVQQFK